European Patent Application EP 4 303 234 A1, published January 10, 2024. Title: Antibody against NKp46 and application of antibody. Applicant: SHANGHAI QILU PHARMACEUTICAL RESEARCH AND DEVELOPMENT CENTRE LTD. The sequence listing filed with the application follows.

SEQUENCE LISTING (152 sequences)

SEQ ID NO: 1 - protein, 304 aa, human
  human NKp46 protein
MSSTLPALLCVGLCLSQRISAQQQTLPKPFIWAEPHFMVPKEKQVTICCQGNYGAVEYQLHFEGSLFAVDRPKPPERINKVKFYIPDMNSRMAGQYSCIYRVGELWSEPSNLLDLVVTEMYDTPTLSVHPGPEVISGEKVTFYCRLDTATSMFLLLKEGRSSHVQRGYGKVQAEFPLGPVTTAHRGTYRCFGSYNNHAWSFPSEPVKLLVTGDIENTSLAPEDPTFPADTWGTYLLTTETGLQKDHALWDHTAQNLLRMGLAFLVLVALVWFLVEDWLSRKRTRERASRASTWEGRRRLNTQTL

SEQ ID NO: 2 - protein, 306 aa, Macaca fascicularis
  Macaca fascicularis NKp46 protein
MSSTLRALLCLGLCLSQRISAPKQTLPKPIIRAESTYMVPKEKQATLCCQGSYGAVEYQLHFEGSLFAVERPKPPERINGVKFHIPDMNSRKAGRYSCIYRVGELWSERSDLLDLVVTEMYDTPTLSVHPGPEVTSGEKVTFYCRLDTATSMFLLLKEGRSRDVQRSYGKVQAEFPMGPVTTAHRGSYRCFGSYNNYAWSFPSEPVKLLVTGDIENTSLAPTDPTFPDSWDTCLLTRETGLQKDLALWDHTAQNLLRMGLAFLVLVALVCLLVEDWLSRKRTREQASRASTWEGRRRLNKHKDSEE

SEQ ID NO: 3 - protein, 241 aa, human
  synthetically generated protein
HHHHHHHHQQQTLPKPFIWAEPHFMVPKEKQVTICCQGNYGAVEYQLHFEGSLFAVDRPKPPERINKVKFYIPDMNSRMAGQYSCIYRVGELWSEPSNLLDLVVTEMYDTPTLSVHPGPEVISGEKVTFYCRLDTATSMFLLLKEGRSSHVQRGYGKVQAEFPLGPVTTAHRGTYRCFGSYNNHAWSFPSEPVKLLVTGDIENTSLAPEDPTFPDTWGTYLLTTETGLQKDHALWDHTAQN

SEQ ID NO: 4 - protein, 241 aa, Macaca fascicularis
  synthetically generated protein
PKQTLPKPIIRAESTYMVPKEKQATLCCQGSYGAVEYQLHFEGSLFAVERPKPPERINGVKFHIPDMNSRKAGRYSCIYRVGELWSERSDLLDLVVTEMYDTPTLSVHPGPEVTSGEKVTFYCRLDTATSMFLLLKEGRSRDVQRSYGKVQAEFPMGPVTTAHRGSYRCFGSYNNYAWSFPSEPVKLLVTGDIENTSLAPTDPTFPDSWDTCLLTRETGLQKDLALWDHTAQNHHHHHHHH

SEQ ID NO: 5 - DNA, 23 bp, Artificial Sequence
  primer
gtcctggctgctcttctacaagg

SEQ ID NO: 6 - DNA, 23 bp, Artificial Sequence
  primer
ggtacgtgctgttgaactgttcc

SEQ ID NO: 7 - DNA, 53 bp, Artificial Sequence
  primer
actcgcggcccagccggccatggccgaggtgcagctggtggagtctgggggag

SEQ ID NO: 8 - DNA, 53 bp, Artificial Sequence
  primer
actcgcggcccagccggccatggcccaggtrcagctggtggagtctgggggag

SEQ ID NO: 9 - DNA, 53 bp, Artificial Sequence
  primer
actcgcggcccagccggccatggccgatgtgcagctggtggagtctgggggag

SEQ ID NO: 10 - DNA, 46 bp, Artificial Sequence
  primer
ggtgttggcctcccgggccactagtgctkgagacrgtgacctgggt

SEQ ID NO: 11 - DNA, 46 bp, Artificial Sequence
  primer
ggtgttggcctcccgggccactagtgctkgagacrgtgaccagggt

SEQ ID NO: 12 - DNA, 46 bp, Artificial Sequence
  primer
ggtgttggcctcccgggccactagttgakgagacrgtgacctgggt

SEQ ID NO: 13 - DNA, 46 bp, Artificial Sequence
  primer
ggtgttggcctcccgggccactagttgakgagacrgtgaccagggt

SEQ ID NO: 14 - protein, 124 aa, Artificial Sequence
  synthetically generated protein
QVQLVESGGGSVQAGGSLTLSCATSGYTYRTDCMGWFRQAPGKEREGLATIYTSDGRTDYANSVKGRFTISQDNAKNTLYLHMNNLKPEDTAIYYCAADPQYGGVCPSGGWNYWGQGTQVTVSS

SEQ ID NO: 15 - protein, 115 aa, Artificial Sequence
  synthetically generated protein
QVQLVESGGGLVQPGGSLRLSCAASGFAFSNYNMFWVRQAPGEGFEWISVINRGGDTADYAASVKGRFTISRDNAKNTLYLQMNSLKTEDTAVYYCARDPLGTTRGQGTLVTVSS

SEQ ID NO: 16 - protein, 122 aa, Artificial Sequence
  synthetically generated protein
DVQLVESGGGSVEAGGSLRLSCAASGYRQRTMGWFRQAPGKAREGVACIYTGPTTTFTDYADSVKGRFTITQDNAKNTVYLQMNSLKPEDTAMYYCAANLAYPLTIIPDTRWGQGTQVTVSS

SEQ ID NO: 17 - protein, 129 aa, Artificial Sequence
  synthetically generated protein
EVQLVESGGGSVQAGGSLRLSCTVSGYTGTIEYMGWGWFRQAPGKEREGVAYINTGGGTSVYDDSVKGRFTISKDDVNLTVYLQMNSLKPEDTAIYYCATGSFFGIWYKVPATQYFHYWGQGTQVTVSS

SEQ ID NO: 18 - protein, 129 aa, Artificial Sequence
  synthetically generated protein
DVQLVESGGGSVQAGGSLRLSCAASGYRSRHYCMGWFRQFPGKERERVALINTGGPTTFYADFVEGRFTISLDNAKNTLSLQMNSLKPEDTAMYYCAAGPPSSDSGSGCYVPEYMYNYWGQGTQVTVSS

SEQ ID NO: 19 - protein, 124 aa, Artificial Sequence
  synthetically generated protein
EVQLVESGGGSVQAGGSLRLSCAASGYTYRTDCMGWFRQAPGKEREGLATIYTSDGRTAYADSVKGRFTISQDNAKNTLYLDMNTLKPEDTAMYYCAADLQYGGSCPSGGWKYWGQGTLVTVSS

SEQ ID NO: 20 - protein, 135 aa, Artificial Sequence
  synthetically generated protein
EVQLVESGGGSVQAGGSLRLSCAVSRGSMASTGCMAWFRQTPGKEREAVAIINISGTTRYTDSVKGRFTIAQDSAKNTLTLQMNSLKPEDTGMYYCAATQNPRTVGRGYCTGDYFQVGGGGYSFWGQGTQVTVSS

SEQ ID NO: 21 - protein, 123 aa, Artificial Sequence
  synthetically generated protein
QVQLVESGGGSVQAGGSLRLSCAASGYTYRRYCMAWFRQGPGKEREGVACLDRDGSTTYADSVKGRFTISRDNANDTLYLQMNSLKPEDTALYRCAAAQPGDCWGRRYGFNTWGQGTLVTVSS

SEQ ID NO: 22 - protein, 126 aa, Artificial Sequence
  synthetically generated protein
DVQLVESGGGSVQAGGSLRLSCAPSPYSANSFSMAWFRQVPGKEREGIACIQAESGSTNVAPSVKGRFSISQDNAKNTLYLQMNNLKPEDTAMYYCAAFKRNVGGCELRPEHWRFWGQGTLVTVSS

SEQ ID NO: 23 - protein, 117 aa, Artificial Sequence
  synthetically generated protein
QVQLVESGGGSVQTGGSLRLSCTAPGFTTDSCGMDWYRQAAGKQREWVSRIRPDGRTDYVESVKGRFTISEDKAKYTVYLQMNSLKPEDTAMYSCTTWGLCTAKFRWGQGTQVTVSS

SEQ ID NO: 24 - protein, 131 aa, Artificial Sequence
  synthetically generated protein
DVQLVESGGGSVQAGGSLRLSCAASGYTRSIYYMGWFRQAPGKEREGVAVMHTGGGSTYYTDSVKGRFTISQDNAKNTVYLQMNSLKPEDTAMYYCAASKYLLAFGGVEWILRPAGGWDYWAQGTQVTVSS

SEQ ID NO: 25 - protein, 120 aa, Artificial Sequence
  synthetically generated protein
DVQLVESGGGLVQPGGSLRLSCAISGFTFSIVSMSWVRQAPGKGPERVSWINGDSSNTSYADSVKGRFTISRDNARNMLYLQMNSLKSEDTARYYCTTQNSHYDIRFGYWGQGTQVTVSS

SEQ ID NO: 26 - protein, 127 aa, Artificial Sequence
  synthetically generated protein
DVQLVESGGGLVQAGGSLRLSCAASGRTLSSYAMGWFRQAPGLEREFVAAISRISGDTYSPDSVKGRFTISRDNAKNTLYLQMNSLKPEDTAVYYCAASATPSATNIYTNQYAYGDWGQGTQVTVSS

SEQ ID NO: 27 - protein, 121 aa, Artificial Sequence
  synthetically generated protein
DVQLVESGGGLVQAGGSLRLSCAASGRTFNTIHWFRQAPGKEREFVARIWWIERTTFYAASVKGRFTISRDNAKNMVYLQMNSLKPEDTAVYYCAADARYTGSRRWESDYWGQGTQVTVSS

SEQ ID NO: 28 - protein, 118 aa, Artificial Sequence
  synthetically generated protein
DVQLVESGGGLVQAGGSLRLSCAASGHTESWYRMGWFRQAPGKGREVVGRISGSPGILYYAGSVKGRFTISRDNAKNTLYLQMTNLKPEDTARYYCAADRTGATWDYWGQGTQVTVSS

SEQ ID NO: 29 - protein, 127 aa, Artificial Sequence
  synthetically generated protein
QVQLVESGGGLVQAGDSLRVSCAASGRTFSTYAMGWFRQAPGKEREFVAASSRDGTTTYYADSVKGRFTISRDNAKNTVYLQMNSLKPEDTAVYYCAASRPLSTTQVGIASAWYEYWGQGTQVTVSS

SEQ ID NO: 30 - protein, 127 aa, Artificial Sequence
  synthetically generated protein
QVQLVESGGGLVQPGGSLRLACAASGRTFSTYAMGWFRQAPGKEREFVAAISRNGGTTYYADSVKGRFTISRDNAKNTVYLQMNSLKPEDTAVYYCAASRPLSNTQVGVASAWYEFWGQGTLVTVSS

SEQ ID NO: 31 - protein, 121 aa, Artificial Sequence
  synthetically generated protein
QVQLVESGGGLVQAGGSLRLSCTASGRTFETLHWFRQAPGKEREFVARIWWIGGATFYADSVKGRFTISRDNAKNMVYLQMNSLKPEDTAIYYCAADARYTSNRRWESDYWGQGTQVTVSS

SEQ ID NO: 32 - protein, 124 aa, Artificial Sequence
  synthetically generated protein
QVQLVESGGGQVQAGGSLRLSCVASGRTYSIYGMGWFRQAPGKEREVVAAINWSSGHTYYADSVKGRFTISKDNAKNTHYLQMNSLKPEDTAVYYCAADSIYGLSFTVKDYDYWGQGTLVTVSS

SEQ ID NO: 33 - protein, 121 aa, Artificial Sequence
  synthetically generated protein
QVQLVESGGGMVQAGGSLRLSCAASGRTFNTIHWFRQAPGKEREFVARIWWIGGATFYADSVKGRFTISRDNTENLVYLQMNSLKPEDTAVYYCAADARYTSHGYYESDYWGPGTQVTVSS

SEQ ID NO: 34 - protein, 118 aa, Artificial Sequence
  synthetically generated protein
DVQLVESGGGLVQAGASLRLSCAASGRTESWYRMGWFRQAPGKGREVVARISGDTNIKYYAGSVKGRFTISRDNAKNTLYLQMTNLKPEDTARYYCAADRTGATWDYWGQGTQVTVSS

SEQ ID NO: 35 - protein, 127 aa, Artificial Sequence
  synthetically generated protein
QVQLVESGGGLVQAGDSLRLSCVASGRTFSTYAMGWFRQAPGKEREFVAAISRNADTTYYADSVKGRFTISRDNAKNTVYLQMNSLKPEDTAVYYCAADRYSSNTQVGVARTYYDYWGQGTQVTVSS

SEQ ID NO: 36 - protein, 124 aa, Artificial Sequence
  synthetically generated protein
QVQLVESGGGWVQPGGSLRLSCAASGRTYSIYGMGWFRQAPGKEREIVAAINWNSGHTYYADSVKGRFTISRDNAKNTHYLQMNSLKPEDTAVYYCAADSIIGLSFTVKDYDYWGQGTQVTVSS

SEQ ID NO: 37 - protein, 130 aa, Artificial Sequence
  synthetically generated protein
DVQLVESGGGLVQAGDSLRLSCAVSGRTFSRLPMGWFRQGPGKDREFVAAISWSSSTTYYADSVKGRFFISRDNAKNTAYLQMNNLRLEDTAVYYCAAVGGSLDYSATVVYTAARAYADWGQGTLVTVSS

SEQ ID NO: 38 - protein, 118 aa, Artificial Sequence
  synthetically generated protein
QVQLVESGGGLVQTGGSLRLSCAASGSTSSFYRMGWFRQAPGKEREAVARISSSAGLIYYVDSVKGRFTISRAGAKNTVYLQMNSLKPEDTAVYYCAADRHGTRWDYWGQGTQVTVSS

SEQ ID NO: 39 - protein, 127 aa, Artificial Sequence
  synthetically generated protein
QVQLVESGGGLVQAGGSLRLSCAASGRSFSRYAMGWFRQAPGKERDFVAAISSSGDPTYYADSVKGRFTISRVNAKNTVYLQMNSVNPGDTAVYYCAAGLTARDTTVVVHPNGYSYWGQGTQVTVSS

SEQ ID NO: 40 - protein, 127 aa, Artificial Sequence
  synthetically generated protein
QVQLVESGGGLVQAGGSLRLSCAASGRTFSRYSMGWFRQAPGKEREFVAAISSSGDVTHYADSAKGRFIISRDNAKNTVSLQVNSVNLEDTAVYYCAASLTARATTVTVHPNGYNYWGQGTQVTVSS

SEQ ID NO: 41 - protein, 130 aa, Artificial Sequence
  synthetically generated protein
QVQLVESGGGLVQAGGSLRLLCAASGRTFSRLPMAWFRQGPGKDREFVAAISWSGGSTYYADSMKGRFTISRDNAKNTAYLQMNSLRLEDTAVYYCAAVGDSAPYSATIVYTDARAYAYWGQGTQVTVSS

SEQ ID NO: 42 - protein, 127 aa, Artificial Sequence
  synthetically generated protein
EVQLVESGGGLVQPGGSLRLSCAASGRTSTSYAMGWFRQAPGKEREFVAAINRSGDFPYYADSVKGRFTIFRDNAKNTVYLQMSSVKPEDTGVYFCAAAPRAPATQVVISAFGYEYWGQGTQVTVSS

SEQ ID NO: 43 - protein, 127 aa, Artificial Sequence
  synthetically generated protein
QVQLVESGGGLIQAGGSLRLSCVASERSLTLYAMGWFRQAPGLEREFVAGISRTGDTTYSPDSVKGRFTISRDNAKNVLYLQMNSLKPDDTAVYYCAASATYSATNIYTHQRAYGDWGQGTQVTVSS

SEQ ID NO: 44 - protein, 5 aa, Artificial Sequence
  synthetically generated protein
TDCMG

SEQ ID NO: 45 - protein, 17 aa, Artificial Sequence
  synthetically generated protein
TIYTSDGRTDYANSVKG

SEQ ID NO: 46 - protein, 15 aa, Artificial Sequence
  synthetically generated protein
DPQYGGVCPSGGWNY

SEQ ID NO: 47 - protein, 5 aa, Artificial Sequence
  synthetically generated protein
NYNMF

SEQ ID NO: 48 - protein, 17 aa, Artificial Sequence
  synthetically generated protein
VINRGGDTADYAASVKG

SEQ ID NO: 49 - protein, 6 aa, Artificial Sequence
  synthetically generated protein
DPLGTT

SEQ ID NO: 50 - protein, 3 aa, Artificial Sequence
  synthetically generated protein
TMG

SEQ ID NO: 51 - protein, 19 aa, Artificial Sequence
  synthetically generated protein
CIYTGPTTTFTDYADSVKG

SEQ ID NO: 52 - protein, 13 aa, Artificial Sequence
  synthetically generated protein
NLAYPLTIIPDTR

SEQ ID NO: 53 - protein, 7 aa, Artificial Sequence
  synthetically generated protein
IEYMGWG

SEQ ID NO: 54 - protein, 17 aa, Artificial Sequence
  synthetically generated protein
YINTGGGTSVYDDSVKG

SEQ ID NO: 55 - protein, 18 aa, Artificial Sequence
  synthetically generated protein
GSFFGIWYKVPATQYFHY

SEQ ID NO: 56 - protein, 5 aa, Artificial Sequence
  synthetically generated protein
HYCMG

SEQ ID NO: 57 - protein, 17 aa, Artificial Sequence
  synthetically generated protein
LINTGGPTTFYADFVEG

SEQ ID NO: 58 - protein, 20 aa, Artificial Sequence
  synthetically generated protein
GPPSSDSGSGCYVPEYMYNY

SEQ ID NO: 59 - protein, 5 aa, Artificial Sequence
  synthetically generated protein
TDCMG

SEQ ID NO: 60 - protein, 17 aa, Artificial Sequence
  synthetically generated protein
TIYTSDGRTAYADSVKG

SEQ ID NO: 61 - protein, 15 aa, Artificial Sequence
  synthetically generated protein
DLQYGGSCPSGGWKY

SEQ ID NO: 62 - protein, 5 aa, Artificial Sequence
  synthetically generated protein
TGCMA

SEQ ID NO: 63 - protein, 16 aa, Artificial Sequence
  synthetically generated protein
IINISGTTRYTDSVKG

SEQ ID NO: 64 - protein, 26 aa, Artificial Sequence
  synthetically generated protein
TQNPRTVGRGYCTGDYFQVGGGGYSF

SEQ ID NO: 65 - protein, 5 aa, Artificial Sequence
  synthetically generated protein
RYCMA

SEQ ID NO: 66 - protein, 16 aa, Artificial Sequence
  synthetically generated protein
CLDRDGSTTYADSVKG

SEQ ID NO: 67 - protein, 15 aa, Artificial Sequence
  synthetically generated protein
AQPGDCWGRRYGFNT

SEQ ID NO: 68 - protein, 5 aa, Artificial Sequence
  synthetically generated protein
SFSMA

SEQ ID NO: 69 - protein, 17 aa, Artificial Sequence
  synthetically generated protein
CIQAESGSTNVAPSVKG

SEQ ID NO: 70 - protein, 17 aa, Artificial Sequence
  synthetically generated protein
FKRNVGGCELRPEHWRF

SEQ ID NO: 71 - protein, 5 aa, Artificial Sequence
  synthetically generated protein
SCGMD

SEQ ID NO: 72 - protein, 16 aa, Artificial Sequence
  synthetically generated protein
RIRPDGRTDYVESVKG

SEQ ID NO: 73 - protein, 9 aa, Artificial Sequence
  synthetically generated protein
WGLCTAKFR

SEQ ID NO: 74 - protein, 5 aa, Artificial Sequence
  synthetically generated protein
IYYMG

SEQ ID NO: 75 - protein, 17 aa, Artificial Sequence
  synthetically generated protein
VMHTGGGSTYYTDSVKG

SEQ ID NO: 76 - protein, 22 aa, Artificial Sequence
  synthetically generated protein
SKYLLAFGGVEWILRPAGGWDY

SEQ ID NO: 77 - protein, 5 aa, Artificial Sequence
  synthetically generated protein
IVSMS

SEQ ID NO: 78 - protein, 17 aa, Artificial Sequence
  synthetically generated protein
WINGDSSNTSYADSVKG

SEQ ID NO: 79 - protein, 11 aa, Artificial Sequence
  synthetically generated protein
QNSHYDIRFGY

SEQ ID NO: 80 - protein, 5 aa, Artificial Sequence
  synthetically generated protein
SYAMG

SEQ ID NO: 81 - protein, 17 aa, Artificial Sequence
  synthetically generated protein
AISRISGDTYSPDSVKG

SEQ ID NO: 82 - protein, 18 aa, Artificial Sequence
  synthetically generated protein
SATPSATNIYTNQYAYGD

SEQ ID NO: 83 - protein, 3 aa, Artificial Sequence
  synthetically generated protein
TIH

SEQ ID NO: 84 - protein, 17 aa, Artificial Sequence
  synthetically generated protein
RIWWIERTTFYAASVKG

SEQ ID NO: 85 - protein, 14 aa, Artificial Sequence
  synthetically generated protein
DARYTGSRRWESDY

SEQ ID NO: 86 - protein, 5 aa, Artificial Sequence
  synthetically generated protein
WYRMG

SEQ ID NO: 87 - protein, 17 aa, Artificial Sequence
  synthetically generated protein
RISGSPGILYYAGSVKG

SEQ ID NO: 88 - protein, 9 aa, Artificial Sequence
  synthetically generated protein
DRTGATWDY

SEQ ID NO: 89 - protein, 5 aa, Artificial Sequence
  synthetically generated protein
TYAMG

SEQ ID NO: 90 - protein, 17 aa, Artificial Sequence
  synthetically generated protein
ASSRDGTTTYYADSVKG

SEQ ID NO: 91 - protein, 18 aa, Artificial Sequence
  synthetically generated protein
SRPLSTTQVGIASAWYEY

SEQ ID NO: 92 - protein, 5 aa, Artificial Sequence
  synthetically generated protein
TYAMG

SEQ ID NO: 93 - protein, 17 aa, Artificial Sequence
  synthetically generated protein
AISRNGGTTYYADSVKG

SEQ ID NO: 94 - protein, 18 aa, Artificial Sequence
  synthetically generated protein
SRPLSNTQVGVASAWYEF

SEQ ID NO: 95 - protein, 3 aa, Artificial Sequence
  synthetically generated protein
TLH

SEQ ID NO: 96 - protein, 17 aa, Artificial Sequence
  synthetically generated protein
RIWWIGGATFYADSVKG

SEQ ID NO: 97 - protein, 14 aa, Artificial Sequence
  synthetically generated protein
DARYTSNRRWESDY

SEQ ID NO: 98 - protein, 5 aa, Artificial Sequence
  synthetically generated protein
IYGMG

SEQ ID NO: 99 - protein, 17 aa, Artificial Sequence
  synthetically generated protein
AINWSSGHTYYADSVKG

SEQ ID NO: 100 - protein, 15 aa, Artificial Sequence
  synthetically generated protein
DSIYGLSFTVKDYDY

SEQ ID NO: 101 - protein, 3 aa, Artificial Sequence
  synthetically generated protein
TIH

SEQ ID NO: 102 - protein, 17 aa, Artificial Sequence
  synthetically generated protein
RIWWIGGATFYADSVKG

SEQ ID NO: 103 - protein, 14 aa, Artificial Sequence
  synthetically generated protein
DARYTSHGYYESDY

SEQ ID NO: 104 - protein, 5 aa, Artificial Sequence
  synthetically generated protein
WYRMG

SEQ ID NO: 105 - protein, 17 aa, Artificial Sequence
  synthetically generated protein
RISGDTNIKYYAGSVKG

SEQ ID NO: 106 - protein, 9 aa, Artificial Sequence
  synthetically generated protein
DRTGATWDY

SEQ ID NO: 107 - protein, 5 aa, Artificial Sequence
  synthetically generated protein
TYAMG

SEQ ID NO: 108 - protein, 17 aa, Artificial Sequence
  synthetically generated protein
AISRNADTTYYADSVKG

SEQ ID NO: 109 - protein, 18 aa, Artificial Sequence
  synthetically generated protein
DRYSSNTQVGVARTYYDY

SEQ ID NO: 110 - protein, 5 aa, Artificial Sequence
  synthetically generated protein
IYGMG

SEQ ID NO: 111 - protein, 17 aa, Artificial Sequence
  synthetically generated protein
AINWNSGHTYYADSVKG

SEQ ID NO: 112 - protein, 15 aa, Artificial Sequence
  synthetically generated protein
DSIIGLSFTVKDYDY

SEQ ID NO: 113 - protein, 5 aa, Artificial Sequence
  synthetically generated protein
RLPMG

SEQ ID NO: 114 - protein, 17 aa, Artificial Sequence
  synthetically generated protein
AISWSSSTTYYADSVKG

SEQ ID NO: 115 - protein, 21 aa, Artificial Sequence
  synthetically generated protein
VGGSLDYSATVVYTAARAYAD

SEQ ID NO: 116 - protein, 5 aa, Artificial Sequence
  synthetically generated protein
FYRMG

SEQ ID NO: 117 - protein, 17 aa, Artificial Sequence
  synthetically generated protein
RISSSAGLIYYVDSVKG

SEQ ID NO: 118 - protein, 9 aa, Artificial Sequence
  synthetically generated protein
DRHGTRWDY

SEQ ID NO: 119 - protein, 5 aa, Artificial Sequence
  synthetically generated protein
RYAMG

SEQ ID NO: 120 - protein, 17 aa, Artificial Sequence
  synthetically generated protein
AISSSGDPTYYADSVKG

SEQ ID NO: 121 - protein, 18 aa, Artificial Sequence
  synthetically generated protein
GLTARDTTVVVHPNGYSY

SEQ ID NO: 122 - protein, 5 aa, Artificial Sequence
  synthetically generated protein
RYSMG

SEQ ID NO: 123 - protein, 17 aa, Artificial Sequence
  synthetically generated protein
AISSSGDVTHYADSAKG

SEQ ID NO: 124 - protein, 18 aa, Artificial Sequence
  synthetically generated protein
SLTARATTVTVHPNGYNY

SEQ ID NO: 125 - protein, 5 aa, Artificial Sequence
  synthetically generated protein
RLPMA

SEQ ID NO: 126 - protein, 17 aa, Artificial Sequence
  synthetically generated protein
AISWSGGSTYYADSMKG

SEQ ID NO: 127 - protein, 21 aa, Artificial Sequence
  synthetically generated protein
VGDSAPYSATIVYTDARAYAY

SEQ ID NO: 128 - protein, 5 aa, Artificial Sequence
  synthetically generated protein
SYAMG

SEQ ID NO: 129 - protein, 17 aa, Artificial Sequence
  synthetically generated protein
AINRSGDFPYYADSVKG

SEQ ID NO: 130 - protein, 18 aa, Artificial Sequence
  synthetically generated protein
APRAPATQVVISAFGYEY

SEQ ID NO: 131 - protein, 5 aa, Artificial Sequence
  synthetically generated protein
LYAMG

SEQ ID NO: 132 - protein, 17 aa, Artificial Sequence
  synthetically generated protein
GISRTGDTTYSPDSVKG

SEQ ID NO: 133 - protein, 18 aa, Artificial Sequence
  synthetically generated protein
SATYSATNIYTHQRAYGD

SEQ ID NO: 134 - protein, 233 aa, Artificial Sequence
  synthetically generated protein
  UNSURE (1)..(1): The 'Xaa' at location 1 stands for Gln, Arg, Pro, or Leu.
  UNSURE (2)..(2): The 'Xaa' at location 2 stands for Gln, Arg, Pro, or Leu.
XXGGGGSDKTHTCPPCPAPEAAGGPSVFLFPPKPKDTLMISRTPEVTCVVVDVSHEDPEVKFNWYVDGVEVHNAKTKPREEQYNSTYRVVSVLTVLHQDWLNGKEYKCKVSNKALPAPIEKTISKAKGQPREPQVYTLPPSRDELTKNQVSLTCLVKGFYPSDIAVEWESNGQPENNYKTTPPVLDSDGSFFLYSKLTVDKSRWQQGNVFSCSVMHEALHNHYTQKSLSLSPG

SEQ ID NO: 135 - protein, 126 aa, Artificial Sequence
  synthetically generated protein
EVQLVESGGGLVQPGGSLRLSCAASPYSANSFSMAWVRQAPGKGLEWVSCIQAESGSTNVAPSVKGRFTISRDNSKNTLYLQMNSLRAEDTAVYYCAAFKRNVGGCELRPEHWRFWGQGTLVTVSS

SEQ ID NO: 136 - protein, 126 aa, Artificial Sequence
  synthetically generated protein
EVQLVESGGGLVQPGGSLRLSCAASPYSANSFSMAWFRQAPGKGLEGVACIQAESGSTNVAPSVKGRFTISQDNSKNTLYLQMNSLRAEDTAVYYCAAFKRNVGGCELRPEHWRFWGQGTLVTVSS

SEQ ID NO: 137 - protein, 126 aa, Artificial Sequence
  synthetically generated protein
EVQLVESGGGLVQPGGSLRLSCAPSPYSANSFSMAWFRQAPGKGLEGIACIQAESGSTNVAPSVKGRFTISQDNSKNTLYLQMNSLRAEDTAVYYCAAFKRNVGGCELRPEHWRFWGQGTLVTVSS

SEQ ID NO: 138 - protein, 126 aa, Artificial Sequence
  synthetically generated protein
EVQLVESGGGLVQPGGSLRLSCAASPYSANSFSMAWFRQAPGKGREGVACIQAESGSTNVAPSVKGRFTISQDNSKNTLYLQMNSLRAEDTAVYYCAAFKRNVGGCELRPEHWRFWGQGTLVTVSS

SEQ ID NO: 139 - protein, 126 aa, Artificial Sequence
  synthetically generated protein
EVQLVESGGGLVQPGGSLRLSCAPSPYSANSFSMAWFRQAPGKGREGIACIQAESGSTNVAPSVKGRFTISQDNSKNTLYLQMNSLRAEDTAVYYCAAFKRNVGGCELRPEHWRFWGQGTLVTVSS

SEQ ID NO: 140 - protein, 126 aa, Artificial Sequence
  synthetically generated protein
EVQLVESGGGLVQPGGSLRLSCAPSPYSANSFSMAWFRQAPGKEREGIACIQAESGSTNVAPSVKGRFTISQDNSKNTLYLQMNSLRAEDTAVYYCAAFKRNVGGCELRPEHWRFWGQGTLVTVSS

SEQ ID NO: 141 - protein, 118 aa, Artificial Sequence
  synthetically generated protein
QVQLVESGGGVVQPGRSLRLSCAASGRTESWYRMGWVRQAPGKGLEWVARISGDTNIKYYAGSVKGRFTISRDNSKNTLYLQMSSLRAEDTAVYYCAADRTGATWDYWGQGTLVTVSS

SEQ ID NO: 142 - protein, 118 aa, Artificial Sequence
  synthetically generated protein
QVQLVESGGGVVQPGRSLRLSCAASGRTESWYRMGWFRQAPGKGLEVVARISGDTNIKYYAGSVKGRFTISRDNSKNTLYLQMSSLRAEDTAVYYCAADRTGATWDYWGQGTLVTVSS

SEQ ID NO: 143 - protein, 118 aa, Artificial Sequence
  synthetically generated protein
QVQLVESGGGVVQPGRSLRLSCAASGRTESWYRMGWFRQAPGKGREVVARISGDTNIKYYAGSVKGRFTISRDNSKNTLYLQMSSLRAEDTAVYYCAADRTGATWDYWGQGTLVTVSS

SEQ ID NO: 144 - protein, 118 aa, Artificial Sequence
  synthetically generated protein
DVQLVESGGGVVQPGRSLRLSCAASGRTESWYRMGWFRQAPGKGREVVARISGDTNIKYYAGSVKGRFTISRDNSKNTLYLQMSSLRAEDTAVYYCAADRTGATWDYWGQGTLVTVSS

SEQ ID NO: 145 - protein, 130 aa, Artificial Sequence
  synthetically generated protein
EVQLVESGGGLVQPGGSLRLSCAASGRTFSRLPMGWVRQAPGKGLEWVSAISWSSSTTYYADSVKGRFTISRDNSKNTLYLQMNSLRAEDTAVYYCAAVGGSLDYSATVVYTAARAYADWGQGTLVTVSS

SEQ ID NO: 146 - protein, 130 aa, Artificial Sequence
  synthetically generated protein
EVQLVESGGGLVQPGGSLRLSCAVSGRTFSRLPMGWFRQAPGKGLEFVAAISWSSSTTYYADSVKGRFTISRDNSKNTAYLQMNSLRAEDTAVYYCAAVGGSLDYSATVVYTAARAYADWGQGTLVTVSS

SEQ ID NO: 147 - protein, 130 aa, Artificial Sequence
  synthetically generated protein
EVQLVESGGGLVQPGGSLRLSCAVSGRTFSRLPMGWFRQAPGKGREFVAAISWSSSTTYYADSVKGRFTISRDNSKNTAYLQMNSLRAEDTAVYYCAAVGGSLDYSATVVYTAARAYADWGQGTLVTVSS

SEQ ID NO: 148 - protein, 130 aa, Artificial Sequence
  synthetically generated protein
EVQLVESGGGLVQPGGSLRLSCAVSGRTFSRLPMGWFRQAPGKDREFVAAISWSSSTTYYADSVKGRFTISRDNSKNTAYLQMNSLRAEDTAVYYCAAVGGSLDYSATVVYTAARAYADWGQGTLVTVSS

SEQ ID NO: 149 - protein, 130 aa, Artificial Sequence
  synthetically generated protein
EVQLVESGGGLVQPGGSLRLSCAASGRTFSRLPMAWVRQAPGKGLEWVSAISWSGGSTYYADSMKGRFTISRDNSKNTLYLQMNSLRAEDTAVYYCAAVGDSAPYSATIVYTDARAYAYWGQGTLVTVSS

SEQ ID NO: 150 - protein, 130 aa, Artificial Sequence
  synthetically generated protein
EVQLVESGGGLVQPGGSLRLSCAASGRTFSRLPMAWFRQAPGKGLEFVAAISWSGGSTYYADSMKGRFTISRDNSKNTAYLQMNSLRAEDTAVYYCAAVGDSAPYSATIVYTDARAYAYWGQGTLVTVSS

SEQ ID NO: 151 - protein, 130 aa, Artificial Sequence
  synthetically generated protein
EVQLVESGGGLVQPGGSLRLSCAASGRTFSRLPMAWFRQAPGKGREFVAAISWSGGSTYYADSMKGRFTISRDNSKNTAYLQMNSLRAEDTAVYYCAAVGDSAPYSATIVYTDARAYAYWGQGTLVTVSS

SEQ ID NO: 152 - protein, 130 aa, Artificial Sequence
  synthetically generated protein
EVQLVESGGGLVQPGGSLRLSCAASGRTFSRLPMAWFRQAPGKDREFVAAISWSGGSTYYADSMKGRFTISRDNSKNTAYLQMNSLRAEDTAVYYCAAVGDSAPYSATIVYTDARAYAYWGQGTLVTVSS